European Patent Specification EP 3 694 536 B1, published August 27, 2025. Title: A Cell-Based Seeding Assay for Huntingtin Aggregation. Applicant: The Regents of the University of California Yang, Xiangdong W. Lee, Chung-Ying Wang, Nan. The sequence listing filed with the application follows.

SEQUENCE LISTING (6 sequences)

SEQ ID NO: 1 - DNA, 1065 bp, Artificial Sequence
  Chemically Synthesized, HTTex1-46Q-EGFP nucleic acid sequence
atggcgaccctggaaaagctgatgaaggccttcgagtccctcaaaagcttccaacagcagcaacagcaacaacagcagcaacagcaacaacagcagcaacagcaacaacagcagcaacagcagcaacagcaacaacagcagcaacagcaacaacagcagcaacagcaacaacagcagcaacagcaacaaccgccaccacctccccctccacccccacctcctcaacttcctcaacctcctccacaggcacagcctctgctgcctcagccacaacctcctccacctccacctccacctcctccaggcccagctgtggctgaggagcctctgcaccgacctggatccctggtgagcaagggcgaggagctgttcaccggggtggtgcccatcctggtcgagctggacggcgacgtaaacggccacaagttcagcgtgtccggcgagggcgagggcgatgccacctacggcaagctgaccctgaagttcatctgcaccaccggcaagctgcccgtgccctggcccaccctcgtgaccaccctgacctacggcgtgcagtgcttcagccgctaccccgaccacatgaagcagcacgacttcttcaagtccgccatgcccgaaggctacgtccaggagcgcaccatcttcttcaaggacgacggcaactacaagacccgcgccgaggtgaagttcgagggcgacaccctggtgaaccgcatcgagctgaagggcatcgacttcaaggaggacggcaacatcctggggcacaagctggagtacaactacaacagccacaacgtctatatcatggccgacaagcagaagaacggcatcaaggtgaacttcaagatccgccacaacatcgaggacggcagcgtgcagctcgccgaccactaccagcagaacacccccatcggcgacggccccgtgctgctgcccgacaaccactacctgagcacccagtccgccctgagcaaagaccccaacgagaagcgcgatcacatggtcctgctggagttcgtgaccgccgccgggatcactctcggcatggacgagctgtacaagtaa

SEQ ID NO: 2 - protein, 354 aa, Artificial Sequence
  Chemically Synthesized, HTTex1-46Q-EGFP amino acid sequence
MATLEKLMKAFESLKSFQQQQQQQQQQQQQQQQQQQQQQQQQQQQQQQQQQQQQQQQQQQQQQPPPPPPPPPPPQLPQPPPQAQPLLPQPQPPPPPPPPPPGPAVAEEPLHRPGSLVSKGEELFTGVVPILVELDGDVNGHKFSVSGEGEGDATYGKLTLKFICTTGKLPVPWPTLVTTLTYGVQCFSRYPDHMKQHDFFKSAMPEGYVQERTIFFKDDGNYKTRAEVKFEGDTLVNRIELKGIDFKEDGNILGHKLEYNYNSHNVYIMADKQKNGIKVNFKIRHNIEDGSVQLADHYQQNTPIGDGPVLLPDNHYLSTQSALSKDPNEKRDHMVLLEFVTAAGITLGMDELYK

SEQ ID NO: 3 - DNA, 1017 bp, Artificial Sequence
  Chemically Synthesized, HTTex1-46Q-EGFP nucleic acid sequence lacking encoding sequence for residues 2-16 of SEQ ID NO:2 (N17)
atgcaacagcagcaacagcaacaacagcagcaacagcaacaacagcagcaacagcaacaacagcagcaacagcagcaacagcaacaacagcagcaacagcaacaacagcagcaacagcaacaacagcagcaacagcaacaaccgccaccacctccccctccacccccacctcctcaacttcctcaacctcctccacaggcacagcctctgctgcctcagccacaacctcctccacctccacctccacctcctccaggcccagctgtggctgaggagcctctgcaccgacctggatccctggtgagcaagggcgaggagctgttcaccggggtggtgcccatcctggtcgagctggacggcgacgtaaacggccacaagttcagcgtgtccggcgagggcgagggcgatgccacctacggcaagctgaccctgaagttcatctgcaccaccggcaagctgcccgtgccctggcccaccctcgtgaccaccctgacctacggcgtgcagtgcttcagccgctaccccgaccacatgaagcagcacgacttcttcaagtccgccatgcccgaaggctacgtccaggagcgcaccatcttcttcaaggacgacggcaactacaagacccgcgccgaggtgaagttcgagggcgacaccctggtgaaccgcatcgagctgaagggcatcgacttcaaggaggacggcaacatcctggggcacaagctggagtacaactacaacagccacaacgtctatatcatggccgacaagcagaagaacggcatcaaggtgaacttcaagatccgccacaacatcgaggacggcagcgtgcagctcgccgaccactaccagcagaacacccccatcggcgacggccccgtgctgctgcccgacaaccactacctgagcacccagtccgccctgagcaaagaccccaacgagaagcgcgatcacatggtcctgctggagttcgtgaccgccgccgggatcactctcggcatggacgagctgtacaagtaa

SEQ ID NO: 4 - protein, 338 aa, Artificial Sequence
  Chemically Synthesized, HTTex1-46Q-EGFP amino acid sequence lacking sequence for residues 2-16 of SEQ ID NO:2 (N17)
MQQQQQQQQQQQQQQQQQQQQQQQQQQQQQQQQQQQQQQQQQQQQQQPPPPPPPPPPPQLPQPPPQAQPLLPQPQPPPPPPPPPPGPAVAEEPLHRPGSLVSKGEELFTGVVPILVELDGDVNGHKFSVSGEGEGDATYGKLTLKFICTTGKLPVPWPTLVTTLTYGVQCFSRYPDHMKQHDFFKSAMPEGYVQERTIFFKDDGNYKTRAEVKFEGDTLVNRIELKGIDFKEDGNILGHKLEYNYNSHNVYIMADKQKNGIKVNFKIRHNIEDGSVQLADHYQQNTPIGDGPVLLPDNHYLSTQSALSKDPNEKRDHMVLLEFVTAAGITLGMDELYK

SEQ ID NO: 5 - DNA, 297 bp, Artificial Sequence
  Chemically Synthesized, nucleic acid sequence for a fragment of exon 1 of HTT encoding a 46 polyQ region and a proline rich region
caacagcagcaacagcaacaacagcagcaacagcaacaacagcagcaacagcaacaacagcagcaacagcagcaacagcaacaacagcagcaacagcaacaacagcagcaacagcaacaacagcagcaacagcaacaaccgccaccacctccccctccacccccacctcctcaacttcctcaacctcctccacaggcacagcctctgctgcctcagccacaacctcctccacctccacctccacctcctccaggcccagctgtggctgaggagcctctgcaccgacctggatccctg

SEQ ID NO: 6 - protein, 99 aa, Artificial Sequence
  Chemically Synthesized, amino acid sequence for a fragment of exon 1 of HTT comprising a 46 polyQ region and a proline rich region
QQQQQQQQQQQQQQQQQQQQQQQQQQQQQQQQQQQQQQQQQQQQQQPPPPPPPPPPPQLPQPPPQAQPLLPQPQPPPPPPPPPPGPAVAEEPLHRPGSL